European Patent Application EP 4 219 556 A2, published August 2, 2023. Title: HUMAN MONOCLONAL ANTIBODIES SPECIFIC FOR FLT3 AND USES THEREOF. Applicant: THE UNITED STATES OF AMERICA, AS REPRESENTED BY THE SECRETARY, DEPARTMENT OF HEALTH AND HUMAN SERVICES. Application EP. The sequence listing filed with the application follows.

SEQUENCE LISTING (20 sequences)

SEQ ID NO: 1 - protein, 116 aa, synthetic construct
  REGION 1..116: note = Synthetic polypeptide
EVQLVESGGGLVQPGGSLRLSCAASGFTFSSYGMHWVRQAPGKGLEWVAVISYDGSNKYYADSVKGRFTISRDNSKNTLYLQMNSLRAEDTAVYYCANLAPWAAYWGQGTLVTVSS

SEQ ID NO: 2 - protein, 112 aa, synthetic construct
  REGION 1..112: note = Synthetic polypeptide
EIVLTQSPLSLPVTPGEPASISCRSSQSLLHSNGYNYLDWYLQKPGQSPQLLIYLGSNRASGVPDRFSGSGSGTDFTLKISRVEAEDVGVYYCMQALQTPHTFGQGTKLEIK

SEQ ID NO: 3 - DNA, 729 bp, synthetic construct
  misc_feature 1..729: note = Synthetic polynucleotide
  source 1..729: mol_type = other DNA
gaggtgcagctggtggagtctgggggaggcttggtccagcctggggggtccctgagactctcctgtgcagcctctggattcaccttcagtagctatggcatgcactgggtccgccaggctccaggcaaggggctggagtgggtggcagttatatcatatgacggaagtaataaatactatgcagactccgtgaagggccgattcaccatctccagagacaattccaagaacacgctgtatctgcagatgaacagcctgagagctgaggacacggctgtgtattactgtgcgaacctcgccccgtgggctgcctactggggccagggaaccctggtcaccgtctcctcaggtggaggcggttcaggcggaggtggctctggcggtggcggatcggaaattgtgctgactcagtctccactctccctgcccgtcacccctggagagccggcctccatctcctgcaggtctagtcagagcctcctgcatagtaatggatacaactatttggattggtacctgcagaagccagggcagtctccacagctcctgatctatttgggttctaatcgggcctccggggtccctgacaggttcagtggcagtggatcaggcacagattttacactgaaaatcagcagagtggaggctgaggatgttggggtctattactgcatgcaagctctacaaactcctcacacttttggccaggggaccaaactggagatcaaa

SEQ ID NO: 4 - protein, 243 aa, synthetic construct
  REGION 1..243: note = Synthetic polypeptide
EVQLVESGGGLVQPGGSLRLSCAASGFTFSSYGMHWVRQAPGKGLEWVAVISYDGSNKYYADSVKGRFTISRDNSKNTLYLQMNSLRAEDTAVYYCANLAPWAAYWGQGTLVTVSSGGGGSGGGGSGGGGSEIVLTQSPLSLPVTPGEPASISCRSSQSLLHSNGYNYLDWYLQKPGQSPQLLIYLGSNRASGVPDRFSGSGSGTDFTLKISRVEAEDVGVYYCMQALQTPHTFGQGTKLEIK

SEQ ID NO: 5 - protein, 116 aa, synthetic construct
  REGION 1..116: note = Synthetic polypeptide
EVQLVESGGGVVQPGGSLRLSCAASGFTFSSYGMHWVRQAPGKGLEWVAVISYDGSNKYYADSVKGRFTISRDNSKNTLYLQMNSLRAEDTAVYYCANLAPWAAYWGQGTLVTVSS

SEQ ID NO: 6 - protein, 112 aa, synthetic construct
  REGION 1..112: note = Synthetic polypeptide
DVVMTQSPLSLPVTPGEPASISCRSSQSLLHSNGYNYLDWYLQKPGQSPQLLIYLGSNRASGVPDRFSGSGSGTDFTLKISRVEAEDVGVYYCMQALQTPLTFGGGTKVEIK

SEQ ID NO: 7 - DNA, 729 bp, synthetic construct
  misc_feature 1..729: note = Synthetic polynucleotide
  source 1..729: mol_type = other DNA
gaggtgcagctggtggagtctgggggaggcgtggtccagcctggggggtccctgagactctcctgtgcagcctctggattcaccttcagtagctatggcatgcactgggtccgccaggctccaggcaaggggctggagtgggtggcagttatatcatatgatggaagtaataaatactatgcagactccgtgaagggccgattcaccatctccagagacaattccaagaacacgctgtatctgcaaatgaacagcctgagagctgaggacacggctgtgtattactgtgcgaacctcgccccgtgggctgcctactggggccagggaaccctggtcaccgtctcctcaggtggaggcggttcaggcggaggtggctctggcggtggcggatcggatgttgtgatgactcagtctccactctccctgcccgtcacccctggagagccggcctccatctcctgcaggtctagtcagagcctcctgcatagtaatggatacaactatttggattggtacctgcagaagccagggcagtctccacagctcctgatctatttgggttctaatcgggcctccggggtccctgacaggttcagtggcagtggatcaggcacagattttacactgaaaatcagcagagtggaggctgaggatgttggggtttattactgcatgcaagctctacaaactcctctcactttcggcggagggaccaaggtggagatcaaa

SEQ ID NO: 8 - protein, 243 aa, synthetic construct
  REGION 1..243: note = Synthetic polypeptide
EVQLVESGGGVVQPGGSLRLSCAASGFTFSSYGMHWVRQAPGKGLEWVAVISYDGSNKYYADSVKGRFTISRDNSKNTLYLQMNSLRAEDTAVYYCANLAPWAAYWGQGTLVTVSSGGGGSGGGGSGGGGSDVVMTQSPLSLPVTPGEPASISCRSSQSLLHSNGYNYLDWYLQKPGQSPQLLIYLGSNRASGVPDRFSGSGSGTDFTLKISRVEAEDVGVYYCMQALQTPLTFGGGTKVEIK

SEQ ID NO: 9 - protein, 117 aa, synthetic construct
  REGION 1..117: note = Synthetic polypeptide
QVQLQESGPGLVKPSQTLSLTCTVSGGSISSSGYYWSWVRQSPGKGLEWIGEIYQSGNTNYNPSLKSRVTISVDKPKNQLSLKLGSVTAADTAVYYCARGGSYYDYWGQGTLVTVSS

SEQ ID NO: 10 - protein, 110 aa, synthetic construct
  REGION 1..110: note = Synthetic polypeptide
QSVVTQPPSVSAAPGQKVTISCSGSNSNIGNNYVSWYQQLPGTAPKVLIYDNNVRPSGIPDRFSGSKSGTSATLGITGLQTGDEADYYCETWDSSLNVGMFGGGTQLIVL

SEQ ID NO: 11 - DNA, 726 bp, synthetic construct
  misc_feature 1..726: note = Synthetic polynucleotide
  source 1..726: mol_type = other DNA
caggtgcagctgcaggagtcgggcccaggactagtgaagccttcacagaccctgtccctcacctgcactgtctctggtggctccatcagcagtagtggttactactggagctgggtccgccagtccccagggaaggggctggagtggattggggaaatctatcaaagtgggaacaccaactacaacccgtccctcaagagtcgagtcaccatatcagtagacaagcccaagaaccagctctccctgaagctgggctctgtgaccgccgcggacacggccgtatattactgtgcgagaggtgggagctactacgactactggggccagggaaccctggtcaccgtctcctcaggtggaggcggttcaggcggaggtggctctggcggtggcggatcgcagtctgtcgtgacgcagccgccctcagtgtctgcggccccgggacagaaggtcaccatctcctgctctggaagcaactccaacattggaaataattatgtatcgtggtaccagcaactcccgggaacagcccccaaagtcctcatttatgacaataatgttcgaccctcagggattcctgatcgattctctggctccaagtcaggcacgtcagccaccctgggcatcaccggactccagactggggacgaggccgattattactgcgaaacatgggatagcagcctgaatgttgggatgttcggcggaggcacccagctgatcgtcctc

SEQ ID NO: 12 - protein, 242 aa, synthetic construct
  REGION 1..242: note = Synthetic polypeptide
QVQLQESGPGLVKPSQTLSLTCTVSGGSISSSGYYWSWVRQSPGKGLEWIGEIYQSGNTNYNPSLKSRVTISVDKPKNQLSLKLGSVTAADTAVYYCARGGSYYDYWGQGTLVTVSSGGGGSGGGGSGGGGSQSVVTQPPSVSAAPGQKVTISCSGSNSNIGNNYVSWYQQLPGTAPKVLIYDNNVRPSGIPDRFSGSKSGTSATLGITGLQTGDEADYYCETWDSSLNVGMFGGGTQLIVL

SEQ ID NO: 13 - protein, 118 aa, synthetic construct
  REGION 1..118: note = Synthetic polypeptide
EVQLVQSGGGLVQPGGSLRLSCAASGFTFSSYAMSWVRQAPGKGLEWVSGISWNSGSIGYADSVKGRFTISRDNAKNSLYLQMNSLRAEDTALYYCAKVGGGGAFDIWGQGTMVTVSS

SEQ ID NO: 14 - protein, 109 aa, synthetic construct
  REGION 1..109: note = Synthetic polypeptide
QSVLTQPPSVSAAPGQKVTISCSGSSSSIGDNYVSWYQQVPGTAPKLLIYGNNKRPSGIPDRLSGSKSGTSATLGITGLQTGDEADYYCGTWDNSLGGVFGGGTKLTVL

SEQ ID NO: 15 - DNA, 726 bp, synthetic construct
  misc_feature 1..726: note = Synthetic polynucleotide
  source 1..726: mol_type = other DNA
gaggtgcagctggtgcagtctgggggaggcttggtacagcctggggggtccctgagactctcctgtgcggcctctggattcacctttagcagctatgccatgagctgggtccgccaggctccagggaaggggctggagtgggtctcaggtattagttggaatagtggtagcataggctatgcggactctgtgaagggccgattcaccatctccagagacaacgccaagaactccctgtatctgcaaatgaacagtctgagagctgaggacacggccttgtattactgtgcaaaagttggtgggggtggggcttttgatatctggggccaagggacaatggtcaccgtctcttcaggtggaggcggttcaggcggaggtggctctggcggtggcggatcgcagtctgtgctgacgcagccgccctcagtgtctgcggccccaggacagaaggtcaccatctcctgctctggaagcagctccagcattggggataattatgtatcctggtaccagcaggttcccggaacagcccccaaactcctcatttatggcaataataagcgaccctcagggattcctgaccgactctctggctccaagtctggcacgtcagccaccctgggcatcaccggactccagactggggacgaggccgattattactgcggaacatgggataacagcctggggggggtgttcggcggagggaccaagctgaccgtcctc

SEQ ID NO: 16 - protein, 242 aa, synthetic construct
  REGION 1..242: note = Synthetic polypeptide
EVQLVQSGGGLVQPGGSLRLSCAASGFTFSSYAMSWVRQAPGKGLEWVSGISWNSGSIGYADSVKGRFTISRDNAKNSLYLQMNSLRAEDTALYYCAKVGGGGAFDIWGQGTMVTVSSGGGGSGGGGSGGGGSQSVLTQPPSVSAAPGQKVTISCSGSSSSIGDNYVSWYQQVPGTAPKLLIYGNNKRPSGIPDRLSGSKSGTSATLGITGLQTGDEADYYCGTWDNSLGGVFGGGTKLTVL

SEQ ID NO: 17 - DNA, 360 bp, synthetic construct
  misc_feature 1..360: note = Synthetic polypeptide
  source 1..360: mol_type = other DNA
gaggtgcagctggtggagtctgggggaggcttggtacagcctggagggtccctgagactctcctgtgcagcctctaggttctacttctctgggtatgaaatgagctgggtccgccaggctccagggaagggcctggagtgggtctcagctattagtggtagtggtggtagcacatactacgcagactctgtgaagggccgattcaccatctccagagacaattccaagaacacgctgtatctgcaaatgaacagcctgagagccgaggacacggctgtgtattactgtgcgagaagggtagtgggagctaagctatacttccagcactggggccagggcaccctggtcaccgtctcctca

SEQ ID NO: 18 - protein, 120 aa, synthetic construct
  REGION 1..120: note = Synthetic polypeptide
EVQLVESGGGLVQPGGSLRLSCAASRFYFSGYEMSWVRQAPGKGLEWVSAISGSGGSTYYADSVKGRFTISRDNSKNTLYLQMNSLRAEDTAVYYCARRVVGAKLYFQHWGQGTLVTVSS

SEQ ID NO: 19 - protein, 506 aa, synthetic construct
  REGION 1..506: note = Synthetic polypeptide
MALPVTALLLPLALLLHAARPDYKDDDDKGGGGSGGGGSEVQLVESGGGLVQPGGSLRLSCAASGFTFSSYGMHWVRQAPGKGLEWVAVISYDGSNKYYADSVKGRFTISRDNSKNTLYLQMETNSLRAEDTAVYYCANLAPWAAYWGQGTLVTVSSGGGGSGGGGSEIVLTQSPLSLPVTPGEPASISCRSSQSLLHSNGYNYLDWYLQKPGQSPQLLIYLGSNRASGVPDRFSGSGSGTDFTLKISRVEAEDVGVYYCMQALQTPHTFGQGTKLEIKTSSGTTTPAPRPPTPAPTIASQPLSLRPEACRPAAGGAVHTRGLDFACDIYIWAPLAGTCGVLLLSLVITLYCKRGRKKLLYIFKQPFMRPVQTTQEEDGCSCRFPEEEEGGCELRVKFSRSADAPAYKQGQNQLYNELNLGRREEYDVLDKRRGRDPEMGGKPRRKNPQEGLYNELQKDKMAEAYSEIGMKGERRRGKGHDGLYQGLSTATKDTYDALHMQALPPR

SEQ ID NO: 20 - protein, 14 aa, synthetic construct
  REGION 1..14: note = Synthetic peptide
NYHLENEVARLKKL